European Patent Specification EP 3 247 788 B1, published June 7, 2023. Title: Bacillus strains improving health and performance of production animals. Applicant: Novozymes A/S. The sequence listing filed with the application follows.

SEQUENCE LISTING (13 sequences)

SEQ ID NO: 1 - DNA, 1507 bp, Bacillus amyloliquefaciens
gacgaacgctggcggcgtgcctaatacatgcaagtcgagcggacagatgggagcttgctccctgatgttagcggcggacgggtgagtaacacgtgggtaacctgcctgtaagactgggataactccgggaaaccggggctaataccggatggttgtttgaaccgcatggttcagacataaaaggtggcttcggctaccacttacagatggacccgcggcgcattagctagttggtgaggtaacggctcaccaaggcaacgatgcgtagccgacctgagagggtgatcggccacactgggactgagacacggcccagactcctacgggaggcagcagtagggaatcttccgcaatggacgaaagtctgacggagcaacgccgcgtgagtgatgaaggttttcggatcgtaaagctctgttgttagggaagaacaagtgccgttcaaatagggcggcaccttgacggtacctaaccagaaagccacggctaactacgtgccagcagccgcggtaatacgtaggtggcaagcgttgtccggaattattgggcgtaaagggctcgcaggcggtttcttaagtctgatgtgaaagcccccggctcaaccggggagggtcattggaaactggggaacttgagtgcagaagaggagagtggaattccacgtgtagcggtgaaatgcgtagagatgtggaggaacaccagtggcgaaggcgactctctggtctgtaactgacgctgaggagcgaaagcgtggggagcgaacaggattagataccctggtagtccacgccgtaaacgatgagtgctaagtgttagggggtttccgccccttagtgctgcagctaacgcattaagcactccgcctggggagtacggtcgcaagactgaaactcaaaggaattgacgggggcccgcacaagcggtggagcatgtggtttaattcgaagcaacgcgaagaaccttaccaggtcttgacatcctctgacaatcctagagataggacgtccccttcgggggcagagtgacaggtggtgcatggttgtcgtcagctcgtgtcgtgagatgttgggttaagtcccgcaacgagcgcaacccttgatcttagttgccagcattcagttgggcactctaaggtgactgccggtgacaaaccggaggaaggtggggatgacgtcaaatcatcatgccccttatgacctgggctacacacgtgctacaatgggcagaacaaagggcagcgaaaccgcgaggttaagccaatcccacaaatctgttctcagttcggatcgcagtctgcaactcgactgcgtgaagctggaatcgctagtaatcgcggatcagcatgccgcggtgaatacgttcccgggccttgtacacaccgcccgtcacaccacgagagtttgtaacacccgaagtcggtgaggtaaccttttaggagccagccgccgaaggtgggacagatgattggggtgaagtcgtaacaaggtagccgtatcggaaggtgcgg

SEQ ID NO: 2 - DNA, 1507 bp, Bacillus subtilis
gacgaacgctggcggcgtgcctaatacatgcaagtcgagcggacagatgggagcttgctccctgatgttagcggcggacgggtgagtaacacgtgggtaacctgcctgtaagactgggataactccgggaaaccggggctaataccggatgcttgtttgaaccgcatggttcaaacataaaaggtggcttcggctaccacttacagatggacccgcggcgcattagctagttggtgaggtaacggctcaccaaggcaacgatgcgtagccgacctgagagggtgatcggccacactgggactgagacacggcccagactcctacgggaggcagcagtagggaatcttccgcaatggacgaaagtctgacggagcaacgccgcgtgagtgatgaaggttttcggatcgtaaagctctgttgttagggaagaacaagtaccgttcgaatagggcggtaccttgacggtacctaaccagaaagccacggctaactacgtgccagcagccgcggtaatacgtaggtggcaagcgttgtccggaattattgggcgtaaagggctcgcaggcggtttcttaagtctgatgtgaaagcccccggctcaaccggggagggtcattggaaactggggaacttgagtgcagaagaggagagtggaattccacgtgtagcggtgaaatgcgtagagatgtggaggaacaccagtggcgaaggcgactctctggtctgtaactgacgctgaggagcgaaagcgtggggagcgaacaggattagataccctggtagtccacgccgtaaacgatgagtgctaagtgttagggggtttccgccccttagtgctgcagctaacgcattaagcactccgcctggggagtacggtcgcaagactgaaactcaaaggaattgacgggggcccgcacaagcggtggagcatgtggtttaattcgaagcaacgcgaagaaccttaccaggtcttgacatcctctgacaatcctagagataggacgtccccttcgggggcagagtgacaggtggtgcatggttgtcgtcagctcgtgtcgtgagatgttgggttaagtcccgcaacgagcgcaacccttgatcttagttgccagcattcagttgggcactctaaggtgactgccggtgacaaaccggaggaaggtggggatgacgtcaaatcatcatgccccttatgacctgggctacacacgtgctacaatggacagaacaaagggcagcgaaaccgcgaggttaagccaatcccacaaatctgttctcagttcggatcgcagtctgcaactcgactgcgtgaagctggaatcgctagtaatcgcggatcagcatgccgcggtgaatacgttcccgggccttgtacacaccgcccgtcacaccacgagagtttgtaacacccgaagtcggtgaggtaaccttttaggagccagccgccgaaggtgggacagatgattggggtgaagtcgtaacaaggtagccgtatcggaaggtgcgg

SEQ ID NO: 3 - DNA, 1507 bp, Bacillus subtilis
gacgaacgctggcggcgtgcctaatacatgcaagtcgagcggacagatgggagcttgctccctgatgttagcggcggacgggtgagtaacacgtgggtaacctgcctgtaagactgggataactccgggaaaccggggctaataccggatggttgtttgaaccgcatggttcaaacataaaaggtggcttcggctaccacttacagatggacccgcggcgcattagctagttggtgaggtaacggctcaccaaggcaacgatgcgtagccgacctgagagggtgatcggccacactgggactgagacacggcccagactcctacgggaggcagcagtagggaatcttccgcaatggacgaaagtctgacggagcaacgccgcgtgagtgatgaaggttttcggatcgtaaagctctgttgttagggaagaacaagtaccgttcgaatagggcggtaccttgacggtacctaaccagaaagccacggctaactacgtgccagcagccgcggtaatacgtaggtggcaagcgttgtccggaattattgggcgtaaagggctcgcaggcggtttcttaagtctgatgtgaaagcccccggctcaaccggggagggtcattggaaactggggaacttgagtgcagaagaggagagtggaattccacgtgtagcggtgaaatgcgtagagatgtggaggaacaccagtggcgaaggcgactctctggtctgtaactgacgctgaggagcgaaagcgtggggagcgaacaggattagataccctggtagtccacgccgtaaacgatgagtgctaagtgttagggggtttccgccccttagtgctgcagctaacgcattaagcactccgcctggggagtacggtcgcaagactgaaactcaaaggaattgacgggggcccgcacaagcggtggagcatgtggtttaattcgaagcaacgcgaagaaccttaccaggtcttgacatcctctgacaatcctagagataggacgtccccttcgggggcagagtgacaggtggtgcatggttgtcgtcagctcgtgtcgtgagatgttgggttaagtcccgcaacgagcgcaacccttgatcttagttgccagcattcagttgggcactctaaggtgactgccggtgacaaaccggaggaaggtggggatgacgtcaaatcatcatgccccttatgacctgggctacacacgtgctacaatggacagaacaaagggcagcgaaaccgcgaggttaagccaatcccacaaatctgttctcagttcggatcgcagtctgcaactcgactgcgtgaagctggaatcgctagtaatcgcggatcagcatgccgcggtgaatacgttcccgggccttgtacacaccgcccgtcacaccacgagagtttgtaacacccgaagtcggtgaggtaaccttttaggagccagccgccgaaggtgggacagatgattggggtgaagtcgtaacaaggtagccgtatcggaaggtgcgg

SEQ ID NO: 4 - DNA, 1507 bp, Bacillus amyloliquefaciens
gacgaacgctggcggcgtgcctaatacatgcaagtcgagcggacagatgggagcttgctccctgatgttagcggcggacgggtgagtaacacgtgggtaacctgcctgtaagactgggataactccgggaaaccggggctaataccggatggttgtctgaaccgcatggttcagacataaaaggtggcttcggctaccacttacagatggacccgcggcgcattagctagttggtgaggtaacggctcaccaaggcgacgatgcgtagccgacctgagagggtgatcggccacactgggactgagacacggcccagactcctacgggaggcagcagtagggaatcttccgcaatggacgaaagtctgacggagcaacgccgcgtgagtgatgaaggttttcggatcgtaaagctctgttgttagggaagaacaagtgccgttcaaatagggcggcaccttgacggtacctaaccagaaagccacggctaactacgtgccagcagccgcggtaatacgtaggtggcaagcgttgtccggaattattgggcgtaaagggctcgcaggcggtttcttaagtctgatgtgaaagcccccggctcaaccggggagggtcattggaaactggggaacttgagtgcagaagaggagagtggaattccacgtgtagcggtgaaatgcgtagagatgtggaggaacaccagtggcgaaggcgactctctggtctgtaactgacgctgaggagcgaaagcgtggggagcgaacaggattagataccctggtagtccacgccgtaaacgatgagtgctaagtgttagggggtttccgccccttagtgctgcagctaacgcattaagcactccgcctggggagtacggtcgcaagactgaaactcaaaggaattgacgggggcccgcacaagcggtggagcatgtggtttaattcgaagcaacgcgaagaaccttaccaggtcttgacatcctctgacaatcctagagataggacgtccccttcgggggcagagtgacaggtggtgcatggttgtcgtcagctcgtgtcgtgagatgttgggttaagtcccgcaacgagcgcaacccttgatcttagttgccagcattcagttgggcactctaaggtgactgccggtgacaaaccggaggaaggtggggatgacgtcaaatcatcatgccccttatgacctgggctacacacgtgctacaatggacagaacaaagggcagcgaaaccgcgaggttaagccaatcccacaaatctgttctcagttcggatcgcagtctgcaactcgactgcgtgaagctggaatcgctagtaatcgcggatcagcatgccgcggtgaatacgttcccgggccttgtacacaccgcccgtcacaccacgagagtttgtaacacccgaagtcggtgaggtaacctttaaggagccagccgccgaaggtgggacagatgattggggtgaagtcgtaacaaggtagccgtatcggaaggtgcgg

SEQ ID NO: 5 - DNA, 1472 bp, Bacillus vallismortis
gacgaacgctggcggcgtgcctaatacatgcaagtcgagcggacagatgggagcttgctccctgatgttagcggcggacgggtgagtaacacgtgggtaacctgcctgtaagactgggataactccgggaaaccggggctaataccggatgcttgtttgaaccgcatggttcagacataaaaggtggcttcggctaccacttacagatggacccgcggcgcattagctagttggtgaggtaacggctcaccaaggcgacgatgcgtagccgacctgagagggtgatcggccacactgggactgagacacggcccagactcctacgggaggcagcagtagggaatcttccgcaatggacgaaagtctgacggagcaacgccgcgtgagtgatgaaggttttcggatcgtaaagctctgttgttagggaagaacaagtgccgttcaaatagggcggcaccttgacggtacctaaccagaaagccacggctaactacgtgccagcagccgcggtaatacgtaggtggcaagcgttgtccggaattattgggcgtaaagggctcgcaggcggtttcttaagtctgatgtgaaagcccccggctcaaccggggagggtcattggaaactggggaacttgagtgcagaagaggagagtggaattccacgtgtagcggtgaaatgcgtagagatgtggaggaacaccagtggcgaaggcgactctctggtctgtaactgacgctgaggagcgaaagcgtggggagcgaacaggattagataccctggtagtccacgccgtaaacgatgagtgctaagtgttagggggtttccgccccttagtgctgcagctaacgcattaagcactccgcctggggagtacggtcgcaagactgaaactcaaaggaattgacgggggcccgcacaagcggtggagcatgtggtttaattcgaagcaacgcgaagaaccttaccaggtcttgacatcctctgacaatcctagagataggacgtccccttcgggggcagagtgacaggtggtgcatggttgtcgtcagctcgtgtcgtgagatgttgggttaagtcccgcaacgagcgcaacccttgatcttagttgccagcattcagttgggcactctaaggtgactgccggtgacaaaccggaggaaggtggggatgacgtcaaatcatcatgccccttatgacctgggctacacacgtgctacaatgggcagaacaaagggcagcgaaaccgcgaggttaagccaatcccacaaatctgttctcagttcggatcgcagtctgcaactcgactgcgtgaagctggaatcgctagtaatcgcggatcagcatgccgcggtgaatacgttcccgggccttgtacacaccgcccgtcacaccacgagagtttgtaacacccgaagtcggtgaggtaacctttttggagccagccgccgaaggtgggacagatgattggggtg

SEQ ID NO: 6 - DNA, 1507 bp, Bacillus subtilis; identical to SEQ ID NO: 3

SEQ ID NO: 7 - DNA, 1472 bp, Bacillus amyloliquefaciens; identical to SEQ ID NO: 5

SEQ ID NO: 8 - DNA, 19 bp, Artificial
  PCR primer
gagtttgatcctggctcag

SEQ ID NO: 9 - DNA, 20 bp, Artificial
  PCR primer
agaaaggaggtgatccagcc

SEQ ID NO: 10 - DNA, 21 bp, Artificial
  PCR Primer
atctaatcctgtttgctcccc

SEQ ID NO: 11 - DNA, 15 bp, Artificial
  PCR primer
tacgggaggcagcag

SEQ ID NO: 12 - DNA, 17 bp, Artificial
  PCR Primer
cggtgtgtrcaaggccc

SEQ ID NO: 13 - DNA, 16 bp, Artificial
  PCR Primer
caacgagcgcaaccct